European Patent Specification EP 3 749 957 B1, published June 19, 2024. Title: Elastin Assay. Applicant: Nordic Bioscience A/S. The sequence listing filed with the application follows.

SEQUENCE LISTING (7 sequences)

SEQ ID NO: 1 - protein, 10 aa, Artificial Sequence
  C-Terminus biomarker
LPGGYGLPYT

SEQ ID NO: 2 - protein, 11 aa, Artificial Sequence
  Elongated Peptide
LPGGYGLPYTT

SEQ ID NO: 3 - protein, 9 aa, Artificial Sequence
  Truncated Peptide
LPGGYGLPY

SEQ ID NO: 4 - protein, 13 aa, Artificial Sequence
  SITE 1: KLH attached to N-terminus
  SITE 1: KLH attached to N-terminus
  Immunogenic Peptide
CGGLPGGYGLPYT

SEQ ID NO: 5 - protein, 10 aa, Artificial Sequence
  SITE 1: N-terminal biotinylated
  SITE 1: N-terminal biotinylated
  Biotinylated peptide
LPGGYGLPYT

SEQ ID NO: 6 - protein, 10 aa, Artificial Sequence
  Nonsense peptide
PGGVPGGVFY

SEQ ID NO: 7 - protein, 11 aa, Artificial Sequence
  Non-sense coater
  SITE 11: C-terminal biotinylated
  SITE 11: C-terminal biotinylated
LPGGYGLPYTK